European Patent Specification EP 4 085 067 B1, published September 2, 2026. Title: METHOD FOR DETERMINING 5-METHYLCYTOSINE CONFIGURATIONS IN DNA. Applicant: Technische Universitaet Dortmund. The sequence listing filed with the application follows.

SEQUENCE LISTING (76 sequences)

SEQ ID NO: 1 - protein, 45 aa, Homo sapiens
PALGPGWKRREVFRKSGATCGRSDTYYQSPTGDRIRSKVELTRYL

SEQ ID NO: 2 - protein, 45 aa, Homo sapiens
PALPPGWKKEEVIRKSGLSAGKSDVYYFSPSGKKFRSKPQLARYL

SEQ ID NO: 3 - protein, 45 aa, Homo sapiens
PALPQGWEREEVPRRSGLSAGHRDVFYYSPSGKKFRSKPQLARYL

SEQ ID NO: 4 - protein, 45 aa, Homo sapiens
KSVPCGWERVVKQRLFGKTAGRFDVYFISPQGLKFRSKSSLANYL

SEQ ID NO: 5 - protein, 45 aa, Homo sapiens
PTLPEGWTRKLKQRKSGRSAGKYDVYLINPQGKAFRSKVELIAYF

SEQ ID NO: 6 - protein, 45 aa, Mus musculus
PALGPGWKRRESFRKSGASFGRSDIYYQSPTGEKIRSKVELTRYL

SEQ ID NO: 7 - protein, 45 aa, Mus musculus; identical to SEQ ID NO: 2

SEQ ID NO: 8 - protein, 45 aa, Mus musculus; identical to SEQ ID NO: 3

SEQ ID NO: 9 - protein, 45 aa, Mus musculus
KPVPCGWERVVKQRLSGKTAGKFDVYFISPQGLKFRSKRSLANYL

SEQ ID NO: 10 - protein, 45 aa, Mus musculus; identical to SEQ ID NO: 5

SEQ ID NO: 11 - protein, 45 aa, Rattus norvegicus
PALGPGWKRREAFRKSGASCGRSDIYYRSPTGEKIRSKIELTRYL

SEQ ID NO: 12 - protein, 45 aa, Rattus norvegicus; identical to SEQ ID NO: 2

SEQ ID NO: 13 - protein, 45 aa, Rattus norvegicus; identical to SEQ ID NO: 3

SEQ ID NO: 14 - protein, 45 aa, Pan troglodytes; identical to SEQ ID NO: 4

SEQ ID NO: 15 - protein, 45 aa, Pan troglodytes; identical to SEQ ID NO: 1

SEQ ID NO: 16 - protein, 45 aa, Pan troglodytes; identical to SEQ ID NO: 5

SEQ ID NO: 17 - protein, 45 aa, Pan troglodytes; identical to SEQ ID NO: 5

SEQ ID NO: 18 - protein, 45 aa, Danio rerio
PSLPQGWTRKLKQRKSGRSAGKFDVYLINPEGKAFRSKVELMAYF

SEQ ID NO: 19 - protein, 45 aa, Danio rerio
SALPNGWKMEEVTRKSGLSAGKSDVYYFSPTGKKFRSKPQLVRYL

SEQ ID NO: 20 - protein, 45 aa, Takifugu rubripes
TALPKGWKMEEVTRKSGLSAGKSDVYYFSPSGKKFRSKPQLARYL

SEQ ID NO: 21 - protein, 45 aa, Xenopus laevis
PTLPEGWTRKLKQRKSGRSAGKFDVYLINPNGKAFRSKVELIAYF

SEQ ID NO: 22 - protein, 45 aa, Xenopus laevis
SALPQGWKKEEVTRRSGLSAGKSDVYYYSPSGKKFRSKPQLARYL

SEQ ID NO: 23 - protein, 45 aa, Xenopus laevis
PALPAGWKKEEVIRKSGLSAGKSDVYYYSPNGKKFRSKPQLARYL

SEQ ID NO: 24 - protein, 45 aa, Xenopus laevis
PLLGPGWKRRNVVRKSGATCGHSDTYYRSPAGKKIRSRIELAKYL

SEQ ID NO: 25 - protein, 45 aa, Xenopus laevis
PTLPEGWTRKLKQRKSGRSAGKYDVYLIHPNGKAFRSKVELIAYF

SEQ ID NO: 26 - protein, 45 aa, Gallus gallus; identical to SEQ ID NO: 2

SEQ ID NO: 27 - protein, 45 aa, Strongylocentrotus purpuratus
PGLPAGWKREEVIRKSGLSAGKTDVYYYSPCGKKLRSKPQLARFI

SEQ ID NO: 28 - protein, 46 aa, Strongylocentrotus purpuratus
WPLANGWRRQTIIRQLGPGDRIKGDVIYYAPCGKKLRTYPEVVRYI

SEQ ID NO: 29 - protein, 45 aa, Anopheles gambiae
AALPKGWQREEVLRKTGLSAGKVDVYYYSPTGKKIESKPQLARAL

SEQ ID NO: 30 - protein, 45 aa, Caenorhabditis elegans
LPLQLGWRRQTCVRSIASAGVKGDVSYFAPCGKKLSTYSEVVRYL

SEQ ID NO: 31 - protein, 42 aa, Arabidopsis thaliana
PKTPKGFKRSLVLRKDYSKMDTYYFTPTGKKLRSRNEIAAFV

SEQ ID NO: 32 - protein, 42 aa, Arabidopsis thaliana
PRTPRGFKRSLILRKDYSKMDAYYITPTGKKLKSRNEIAAFI

SEQ ID NO: 33 - protein, 44 aa, Homo sapiens
LPLQHGWRREVRIKKGSHRWQGETWYYGPCGKRMKQFPEVIKYL

SEQ ID NO: 34 - protein, 44 aa, Homo sapiens
IPLEYGWQRETRIRNFGGRLQGEVAYYAPCGKKLRQYPEVIKYL

SEQ ID NO: 35 - protein, 44 aa, Homo sapiens; identical to SEQ ID NO: 33

SEQ ID NO: 36 - protein, 44 aa, Gallus gallus
FPLQHGWRREVRIKRGNHRWQGETWYYGPCGKRMKQFPEVIKYL

SEQ ID NO: 37 - protein, 44 aa, Rattus norvegicus; identical to SEQ ID NO: 33

SEQ ID NO: 38 - protein, 44 aa, Homo sapiens
VPLLYDFRRMTARRRVNRKMGFHVIYKTPCGLCLRTMQEIERYL

SEQ ID NO: 39 - protein, 43 aa, Homo sapiens
LPIKCHFQRRHAKTNSHSSALHVSYKTPCGRSLRNVEEVFRYL

SEQ ID NO: 40 - protein, 44 aa, Homo sapiens; identical to SEQ ID NO: 38

SEQ ID NO: 41 - protein, 43 aa, Homo sapiens
LPIRCHFQRRHAKTNSHSSALHVNYKTPCGRNLRNMEEVFHYL

SEQ ID NO: 42 - protein, 44 aa, Takifugu rubripes
TPLLYDFRRMTGRRKVNRKMSFHVIYKAPCGLCLRNMSEIQHYL

SEQ ID NO: 43 - protein, 44 aa, Xenopus laevis
VPLLYDFRRMTARRRVNRKMGFHVIYKSPCGLSLRTMPEIERYL

SEQ ID NO: 44 - protein, 44 aa, Gallus gallus
IPLLYDFRRMTARRRVNRKMGFHVIYKTPCGLCLRSMAEIERYL

SEQ ID NO: 45 - protein, 44 aa, Rattus norvegicus; identical to SEQ ID NO: 38

SEQ ID NO: 46 - protein, 45 aa, Artificial
  MBD variant of SEQ ID NO:5 (F105)
PTLPEGWTRKLTQRKSGRSAGKYDTTLINPQGKAFRKKVELIAYF

SEQ ID NO: 47 - protein, 45 aa, Artificial
  MBD variant F105-1
PTLPEGWTRKLTQRKSGRSAGKYDTQLINPQGKAFRKKVELIAYF

SEQ ID NO: 48 - protein, 45 aa, Artificial
  MBD variant of SEQ ID NO:5 (F106)
PTLPEGWTRKLTQRKSGRSAGKYDAYLINPQGKAFRNKVELIAYF

SEQ ID NO: 49 - protein, 45 aa, Artificial
  MBD variant F106-1
PTLPEGWTRKLTQRKSGRSAGKYDCYLINPQGKAFRNKVELIAYF

SEQ ID NO: 50 - protein, 45 aa, Artificial
  MBD variant F106-2
PTLPEGWTRKLTQRKSGRSAGKYDAMLINPQGKAFRNKVELIAYF

SEQ ID NO: 51 - protein, 45 aa, Artificial
  MBD variant F260
PTLPEGWTRKLDQRKSGRSAGKYDCYLINPQGKAFRNKVELIAYF

SEQ ID NO: 52 - protein, 45 aa, Artificial
  MBD variant of SEQ ID NO:5 (F271)
PTLPEGWTRKLKQRKSGRSAGKYDCSLINPQGKAFRQKVELIAYF

SEQ ID NO: 53 - protein, 45 aa, Artificial
  MBD variant of SEQ ID NO:5 (F272)
PTLPEGWTRKLAQRKSGRSAGKYDCFLINPQGKAFRRKVELIAYF

SEQ ID NO: 54 - protein, 45 aa, Artificial
  MBD variant F272-1
PTLPEGWTRKLAQRKSGRSAGKYDLMLINPQGKAFRRKVELIAYF

SEQ ID NO: 55 - protein, 45 aa, Artificial
  MBD variant of SEQ ID NO:5 (F273)
PTLPEGWTRKLKQRKSGRSAGKYDLTLINPQGKAFRRKVELIAYF

SEQ ID NO: 56 - protein, 45 aa, Artificial
  MBD variant of SEQ ID NO:5 (F274)
PTLPEGWTRKLVQRKSGRSAGKYDVLLINPQGKAFRRKVELIAYF

SEQ ID NO: 57 - protein, 45 aa, Artificial
  MBD variant of SEQ ID NO:2 (F275)
PALPPGWKKEERIRKSGLSAGKSDVYYFSPSGKKFRVKPQLARYL

SEQ ID NO: 58 - protein, 45 aa, Artificial
  MBD variant F246
PALPQGWEREELPRRSGLSAGHRDYFFYSPSGKKFRFKPQLARYL

SEQ ID NO: 59 - protein, 45 aa, Artificial
  MBD variant F245-B14
PALPPGWKKEELIRKSGLSAGKSDADYFSPDGKKFRSKPQLARYL

SEQ ID NO: 60 - protein, 45 aa, Artificial
  MBD variant F245-B19
PALPPGWKKEEPIRKSGLSAGKSDPVYFSPAGKKFRSKPQLARYL

SEQ ID NO: 61 - protein, 80 aa, Artificial
  MBD variant F246-C1
ERKRWECPALPQGWEREELPRRSGLSAGHRDYFFYSPSGKKFRFKPQLARYLGGSIDLSTFDFRTGKMLMSKMNKSRQRV

SEQ ID NO: 62 - protein, 80 aa, Artificial
  MBD variant F246-A10
ERKRWMCPALPQGWEREELPRRSGLSAGHRDYFFYSPSGKKFRFKPQLARYLGGSMDLSTFDFRTGKMLMSKMNKSRQRV

SEQ ID NO: 63 - protein, 80 aa, Artificial
  MBD variant F245-B23-B3
SGKRMGRPALPPGWKKEELIRKSGLSAGKSDSQYFSPSGEKFRSKPQLARYLGNTVDLSSSDFRTGKMQPSKLQKNKQRL

SEQ ID NO: 64 - protein, 92 aa, Artificial
  MBD variant F248-D13-A2
DRGPMYDDPTHPEGWTRKLAQRKSGRCAGKYDCMLINPQGKAFRNKVELIAYFEKVGDTSLDPNDFDFTVTGRGSPSRREQKPPKKPKSPKA

SEQ ID NO: 65 - protein, 92 aa, Artificial
  MBD variant F106-F22
DRGPMYDDPTPPEGWTRKLTQRKSGRSAGKYDAYLINPHGKAFRNKVELIAYFEKVGDTSLDPNDFDFTVTGRGSPSRRGQKPPKKPKSPKA

SEQ ID NO: 66 - protein, 92 aa, Artificial
  MBD variant F106-C23
YRGPMYDDPTLPEGWTRKLTQRKSGRSAGKYDAYLINPQGKAFRNKVELIAYLGKVGDTSLDPNDFDFTVTGRGSPSRREQKPPKKPKSPKA

SEQ ID NO: 67 - protein, 92 aa, Artificial
  MBD variant F106-1-B9
DRGPMYDDPTLPEGWTRKLTQRKSGRSAGKYDCYLILPQGKALRNKVELIAYFEKVGDTSLDPNDFDFTVTGRGSPSRREQKPPKKPKSPKA

SEQ ID NO: 68 - protein, 80 aa, Artificial
  hMBD2[146-225]
SGKRMDCPALPPGWKKEEVIRKSGLSAGKSDVYYFSPSGKKFRSKPQLARYLGNTVDLSSFDFRTGKMMPSKLQKNKQRL

SEQ ID NO: 69 - protein, 92 aa, Artificial
  hMeCp2[90-181]
DRGPMYDDPTLPEGWTRKLKQRKSGRSAGKYDVYLINPQGKAFRSKVELIAYFEKVGDTSLDPNDFDFTVTGRGSPSRREQKPPKKPKSPKA

SEQ ID NO: 70 - protein, 80 aa, Artificial
  hMBD1[2-81]
AEDWLDCPALGPGWKRREVFRKSGATCGRSDTYYQSPTGDRIRSKVELTRYLGPACDLTLFDFKQGILCYPAPKAHPVAV

SEQ ID NO: 71 - protein, 80 aa, Artificial
  hMBD3[2-81]
ERKRWECPALPQGWEREEVPRRSGLSAGHRDVFYYSPSGKKFRSKPQLARYLGGSMDLSTFDFRTGKMLMSKMNKSRQRV

SEQ ID NO: 72 - protein, 92 aa, Artificial
  hMBD4[76-167]
ATAGTECRKSVPCGWERVVKQRLFGKTAGRFDVYFISPQGLKFRSKSSLANYLHKNGETSLKPEDFDFTVLSKRGIKSRYKDCSMAALTSHL

SEQ ID NO: 73 - protein, 45 aa, Artificial
  MBD variant of SEQ ID NO:5 (L124F)
PTLPEGWTRKLKQRKSGRSAGKYDVYFINPQGKAFRSKVELIAYF

SEQ ID NO: 74 - protein, 45 aa, Artificial
  MBD variant of SEQ ID NO:5 (R133C)
PTLPEGWTRKLKQRKSGRSAGKYDVYLINPQGKAFCSKVELIAYF

SEQ ID NO: 75 - protein, 45 aa, Artificial
  MBD variant of SEQ ID NO:5 (S134C)
PTLPEGWTRKLKQRKSGRSAGKYDVYLINPQGKAFRCKVELIAYF

SEQ ID NO: 76 - protein, 92 aa, Artificial
  Variant of hMeCp2[90-181] (T158M)
DRGPMYDDPTLPEGWTRKLKQRKSGRSAGKYDVYLINPQGKAFRSKVELIAYFEKVGDTSLDPNDFDFMVTGRGSPSRREQKPPKKPKSPKA